European Patent Specification EP 3 233 913 B1, published August 16, 2023. Title: COMPOSITIONS AND METHODS FOR ANTIBODIES TARGETING BMP6. Applicant: NOVARTIS AG. The sequence listing filed with the application follows.

SEQUENCE LISTING (96 sequences)

SEQ ID NO: 1-8 - skipped (8 entries)

SEQ ID NO: 9 - protein, 5 aa, Artificial Sequence
  source: /note="Description of Artificial Sequence: Synthetic peptide"
SYVVH

SEQ ID NO: 10 - protein, 19 aa, Artificial Sequence
  source: /note="Description of Artificial Sequence: Synthetic peptide"
RIKDHKQGYTTAYAASVKG

SEQ ID NO: 11 - protein, 10 aa, Artificial Sequence
  source: /note="Description of Artificial Sequence: Synthetic peptide"
VERSKSGFDN

SEQ ID NO: 12 - protein, 7 aa, Artificial Sequence
  source: /note="Description of Artificial Sequence: Synthetic peptide"
GFTFSSY

SEQ ID NO: 13 - protein, 8 aa, Artificial Sequence
  source: /note="Description of Artificial Sequence: Synthetic peptide"
KDHKQGYT

SEQ ID NO: 14 - protein, 10 aa, Artificial Sequence
  source: /note="Description of Artificial Sequence: Synthetic peptide"
VERSKSGFDN

SEQ ID NO: 15 - protein, 121 aa, Artificial Sequence
  source: /note="Description of Artificial Sequence: Synthetic polypeptide"
QVQLVESGGGLVKPGGSLRLSCAASGFTFSSYVVHWVRQAPGKGLEWVGRIKDHKQGYTTAYAASVKGRFTISRDDSKNTLYLQMNSLKTEDTAVYYCARVERSKSGFDNWGQGTLVTVSS

SEQ ID NO: 16 - DNA, 363 bp, Artificial Sequence
  source: /note="Description of Artificial Sequence: Synthetic polynucleotide"
caggtgcaattggtggaaagcggcggtggcctggtgaaaccaggcggcagcctgcgcctgagctgcgccgcctccggattcaccttttcttcttacgttgttcattgggtgcgccaggccccgggcaaaggtctcgagtgggtgggccgtatcaaagaccacaaacagggctacactactgcttatgccgcctctgtgaaaggccgctttaccattagccgcgatgattcgaaaaacaccctgtatctgcaaatgaacagcctgaaaaccgaagatacggccgtgtattattgcgcgcgtgttgaacgttctaaatctggtttcgataactggggccaaggcaccctggtgactgttagctca

SEQ ID NO: 17 - protein, 451 aa, Artificial Sequence
  source: /note="Description of Artificial Sequence: Synthetic polypeptide"
QVQLVESGGGLVKPGGSLRLSCAASGFTFSSYVVHWVRQAPGKGLEWVGRIKDHKQGYTTAYAASVKGRFTISRDDSKNTLYLQMNSLKTEDTAVYYCARVERSKSGFDNWGQGTLVTVSSASTKGPSVFPLAPSSKSTSGGTAALGCLVKDYFPEPVTVSWNSGALTSGVHTFPAVLQSSGLYSLSSVVTVPSSSLGTQTYICNVNHKPSNTKVDKRVEPKSCDKTHTCPPCPAPELLGGPSVFLFPPKPKDTLMISRTPEVTCVVVDVSHEDPEVKFNWYVDGVEVHNAKTKPREEQYNSTYRVVSVLTVLHQDWLNGKEYKCKVSNKALPAPIEKTISKAKGQPREPQVYTLPPSREEMTKNQVSLTCLVKGFYPSDIAVEWESNGQPENNYKTTPPVLDSDGSFFLYSKLTVDKSRWQQGNVFSCSVMHEALHNHYTQKSLSLSPGK

SEQ ID NO: 18 - DNA, 1353 bp, Artificial Sequence
  source: /note="Description of Artificial Sequence: Synthetic polynucleotide"
caggtgcaattggtggaaagcggcggtggcctggtgaaaccaggcggcagcctgcgcctgagctgcgccgcctccggattcaccttttcttcttacgttgttcattgggtgcgccaggccccgggcaaaggtctcgagtgggtgggccgtatcaaagaccacaaacagggctacactactgcttatgccgcctctgtgaaaggccgctttaccattagccgcgatgattcgaaaaacaccctgtatctgcaaatgaacagcctgaaaaccgaagatacggccgtgtattattgcgcgcgtgttgaacgttctaaatctggtttcgataactggggccaaggcaccctggtgactgttagctcagcctccaccaagggtccatcggtcttccccctggcaccctcctccaagagcacctctgggggcacagcggccctgggctgcctggtcaaggactacttccccgaaccggtgacggtgtcgtggaactcaggcgccctgaccagcggcgtgcacaccttcccggctgtcctacagtcctcaggactctactccctcagcagcgtggtgaccgtgccctccagcagcttgggcacccagacctacatctgcaacgtgaatcacaagcccagcaacaccaaggtggacaagagagttgagcccaaatcttgtgacaaaactcacacatgcccaccgtgcccagcacctgaactcctggggggaccgtcagtcttcctcttccccccaaaacccaaggacaccctcatgatctcccggacccctgaggtcacatgcgtggtggtggacgtgagccacgaagaccctgaggtcaagttcaactggtacgtggacggcgtggaggtgcataatgccaagacaaagccgcgggaggagcagtacaacagcacgtaccgggtggtcagcgtcctcaccgtcctgcaccaggactggctgaatggcaaggagtacaagtgcaaggtctccaacaaagccctcccagcccccatcgagaaaaccatctccaaagccaaagggcagccccgagaaccacaggtgtacaccctgcccccatcccgggaggagatgaccaagaaccaggtcagcctgacctgcctggtcaaaggcttctatcccagcgacatcgccgtggagtgggagagcaatgggcagccggagaacaactacaagaccacgcctcccgtgctggactccgacggctccttcttcctctacagcaagctcaccgtggacaagagcaggtggcagcaggggaacgtcttctcatgctccgtgatgcatgaggctctgcacaaccactacacgcagaagagcctctccctgtctccgggtaaa

SEQ ID NO: 19 - protein, 14 aa, Artificial Sequence
  source: /note="Description of Artificial Sequence: Synthetic peptide"
TGSSSNIGAGYSVH

SEQ ID NO: 20 - protein, 7 aa, Artificial Sequence
  source: /note="Description of Artificial Sequence: Synthetic peptide"
GSSERPS

SEQ ID NO: 21 - protein, 11 aa, Artificial Sequence
  source: /note="Description of Artificial Sequence: Synthetic peptide"
QSWDSSQTLVV

SEQ ID NO: 22 - protein, 10 aa, Artificial Sequence
  source: /note="Description of Artificial Sequence: Synthetic peptide"
SSSNIGAGYS

SEQ ID NO: 23 - protein, 3 aa, Artificial Sequence
  source: /note="Description of Artificial Sequence: Synthetic peptide"
GSS

SEQ ID NO: 24 - protein, 8 aa, Artificial Sequence
  source: /note="Description of Artificial Sequence: Synthetic peptide"
WDSSQTLV

SEQ ID NO: 25 - protein, 111 aa, Artificial Sequence
  source: /note="Description of Artificial Sequence: Synthetic polypeptide"
QSVLTQPPSVSGAPGQRVTISCTGSSSNIGAGYSVHWYQQLPGTAPKLLIYGSSERPSGVPDRFSGSKSGTSASLAITGLQAEDEADYYCQSWDSSQTLVVFGGGTKLTVL

SEQ ID NO: 26 - DNA, 333 bp, Artificial Sequence
  source: /note="Description of Artificial Sequence: Synthetic polynucleotide"
cagagcgtgctgacccagccgccgagcgtgagcggtgcaccgggccagcgcgtgaccattagctgtaccggcagcagcagcaacattggtgctggttactctgtgcattggtaccagcagctgccgggcacggcgccgaaactgctgatctatggtagctctgaacgcccgagcggcgtgccggatcgctttagcggatccaaaagcggcaccagcgccagcctggcgattaccggcctgcaagcagaagacgaagcggattattactgccagtcttgggactcttctcagactctggttgtgtttggcggcggcacgaagttaaccgtccta

SEQ ID NO: 27 - protein, 217 aa, Artificial Sequence
  source: /note="Description of Artificial Sequence: Synthetic polypeptide"
QSVLTQPPSVSGAPGQRVTISCTGSSSNIGAGYSVHWYQQLPGTAPKLLIYGSSERPSGVPDRFSGSKSGTSASLAITGLQAEDEADYYCQSWDSSQTLVVFGGGTKLTVLGQPKAAPSVTLFPPSSEELQANKATLVCLISDFYPGAVTVAWKADSSPVKAGVETTTPSKQSNNKYAASSYLSLTPEQWKSHRSYSCQVTHEGSTVEKTVAPTECS

SEQ ID NO: 28 - DNA, 651 bp, Artificial Sequence
  source: /note="Description of Artificial Sequence: Synthetic polynucleotide"
cagagcgtgctgacccagccgccgagcgtgagcggtgcaccgggccagcgcgtgaccattagctgtaccggcagcagcagcaacattggtgctggttactctgtgcattggtaccagcagctgccgggcacggcgccgaaactgctgatctatggtagctctgaacgcccgagcggcgtgccggatcgctttagcggatccaaaagcggcaccagcgccagcctggcgattaccggcctgcaagcagaagacgaagcggattattactgccagtcttgggactcttctcagactctggttgtgtttggcggcggcacgaagttaaccgtcctaggtcagcccaaggctgccccctcggtcactctgttcccgccctcctctgaggagcttcaagccaacaaggccacactggtgtgtctcataagtgacttctacccgggagccgtgacagtggcctggaaggcagatagcagccccgtcaaggcgggagtggagaccaccacaccctccaaacaaagcaacaacaagtacgcggccagcagctatctgagcctgacgcctgagcagtggaagtcccacagaagctacagctgccaggtcacgcatgaagggagcaccgtggagaagacagtggcccctacagaatgttca

SEQ ID NO: 29 - protein, 5 aa, Artificial Sequence
  source: /note="Description of Artificial Sequence: Synthetic peptide"
SYVVH

SEQ ID NO: 30 - protein, 19 aa, Artificial Sequence
  source: /note="Description of Artificial Sequence: Synthetic peptide"
RIKRESSSYTTMYAAPVKG

SEQ ID NO: 31 - protein, 10 aa, Artificial Sequence
  source: /note="Description of Artificial Sequence: Synthetic peptide"
VERSKSGFDN

SEQ ID NO: 32 - protein, 7 aa, Artificial Sequence
  source: /note="Description of Artificial Sequence: Synthetic peptide"
GFTFSSY

SEQ ID NO: 33 - protein, 8 aa, Artificial Sequence
  source: /note="Description of Artificial Sequence: Synthetic peptide"
KRESSSYT

SEQ ID NO: 34 - protein, 10 aa, Artificial Sequence
  source: /note="Description of Artificial Sequence: Synthetic peptide"
VERSKSGFDN

SEQ ID NO: 35 - protein, 121 aa, Artificial Sequence
  source: /note="Description of Artificial Sequence: Synthetic polypeptide"
QVQLVESGGGLVKPGGSLRLSCAASGFTFSSYVVHWVRQAPGKGLEWVGRIKRESSSYTTMYAAPVKGRFTISRDDSKNTLYLQMNSLKTEDTAVYYCARVERSKSGFDNWGQGTLVTVSS

SEQ ID NO: 36 - DNA, 363 bp, Artificial Sequence
  source: /note="Description of Artificial Sequence: Synthetic polynucleotide"
caggtgcagctggtggaatcaggcggcggactggtcaagcctggcggtagcctgagactgagctgcgctgctagtggcttcaccttctctagctacgtggtgcactgggtcagacaggcccctggtaaaggcctggagtgggtcggacggattaagagagagtcctctagctacactactatgtacgccgctcccgtgaagggccggttcactatctctagggacgactctaagaacaccctgtacctgcagatgaatagcctgaaaaccgaggacaccgccgtctactactgcgctagagtggaacggtctaagtcaggcttcgataactggggtcagggcaccctggtcaccgtgtctagc

SEQ ID NO: 37 - protein, 451 aa, Artificial Sequence
  source: /note="Description of Artificial Sequence: Synthetic polypeptide"
QVQLVESGGGLVKPGGSLRLSCAASGFTFSSYVVHWVRQAPGKGLEWVGRIKRESSSYTTMYAAPVKGRFTISRDDSKNTLYLQMNSLKTEDTAVYYCARVERSKSGFDNWGQGTLVTVSSASTKGPSVFPLAPSSKSTSGGTAALGCLVKDYFPEPVTVSWNSGALTSGVHTFPAVLQSSGLYSLSSVVTVPSSSLGTQTYICNVNHKPSNTKVDKRVEPKSCDKTHTCPPCPAPELLGGPSVFLFPPKPKDTLMISRTPEVTCVVVDVSHEDPEVKFNWYVDGVEVHNAKTKPREEQYNSTYRVVSVLTVLHQDWLNGKEYKCKVSNKALPAPIEKTISKAKGQPREPQVYTLPPSREEMTKNQVSLTCLVKGFYPSDIAVEWESNGQPENNYKTTPPVLDSDGSFFLYSKLTVDKSRWQQGNVFSCSVMHEALHNHYTQKSLSLSPGK

SEQ ID NO: 38 - DNA, 1353 bp, Artificial Sequence
  source: /note="Description of Artificial Sequence: Synthetic polynucleotide"
caggtgcagctggtggaatcaggcggcggactggtcaagcctggcggtagcctgagactgagctgcgctgctagtggcttcaccttctctagctacgtggtgcactgggtcagacaggcccctggtaaaggcctggagtgggtcggacggattaagagagagtcctctagctacactactatgtacgccgctcccgtgaagggccggttcactatctctagggacgactctaagaacaccctgtacctgcagatgaatagcctgaaaaccgaggacaccgccgtctactactgcgctagagtggaacggtctaagtcaggcttcgataactggggtcagggcaccctggtcaccgtgtctagcgctagcactaagggcccaagtgtgtttcccctggcccccagcagcaagtctacttccggcggaactgctgccctgggttgcctggtgaaggactacttccccgagcccgtgacagtgtcctggaactctggggctctgacttccggcgtgcacaccttccccgccgtgctgcagagcagcggcctgtacagcctgagcagcgtggtgacagtgccctccagctctctgggaacccagacctatatctgcaacgtgaaccacaagcccagcaacaccaaggtggacaagagagtggagcccaagagctgcgacaagacccacacctgccccccctgcccagctccagaactgctgggagggccttccgtgttcctgttcccccccaagcccaaggacaccctgatgatcagcaggacccccgaggtgacctgcgtggtggtggacgtgtcccacgaggacccagaggtgaagttcaactggtacgtggacggcgtggaggtgcacaacgccaagaccaagcccagagaggagcagtacaacagcacctacagggtggtgtccgtgctgaccgtgctgcaccaggactggctgaacggcaaagaatacaagtgcaaagtctccaacaaggccctgccagccccaatcgaaaagacaatcagcaaggccaagggccagccacgggagccccaggtgtacaccctgccccccagccgggaggagatgaccaagaaccaggtgtccctgacctgtctggtgaagggcttctaccccagcgatatcgccgtggagtgggagagcaacggccagcccgagaacaactacaagaccacccccccagtgctggacagcgacggcagcttcttcctgtacagcaagctgaccgtggacaagtccaggtggcagcagggcaacgtgttcagctgcagcgtgatgcacgaggccctgcacaaccactacacccagaagtccctgagcctgagccccggcaag

SEQ ID NO: 39 - protein, 14 aa, Artificial Sequence
  source: /note="Description of Artificial Sequence: Synthetic peptide"
TGSSSNIGAGYSVH

SEQ ID NO: 40 - protein, 7 aa, Artificial Sequence
  source: /note="Description of Artificial Sequence: Synthetic peptide"
GQSERPS

SEQ ID NO: 41 - protein, 11 aa, Artificial Sequence
  source: /note="Description of Artificial Sequence: Synthetic peptide"
QSWDSSQTLVV

SEQ ID NO: 42 - protein, 10 aa, Artificial Sequence
  source: /note="Description of Artificial Sequence: Synthetic peptide"
SSSNIGAGYS

SEQ ID NO: 43 - protein, 3 aa, Artificial Sequence
  source: /note="Description of Artificial Sequence: Synthetic peptide"
GQS

SEQ ID NO: 44 - protein, 8 aa, Artificial Sequence
  source: /note="Description of Artificial Sequence: Synthetic peptide"
WDSSQTLV

SEQ ID NO: 45 - protein, 111 aa, Artificial Sequence
  source: /note="Description of Artificial Sequence: Synthetic polypeptide"
QSVLTQPPSVSGAPGQRVTISCTGSSSNIGAGYSVHWYQQLPGTAPKLLIYGQSERPSGVPDRFSGSKSGTSASLAITGLQAEDEADYYCQSWDSSQTLVVFGGGTKLTVL

SEQ ID NO: 46 - DNA, 333 bp, Artificial Sequence
  source: /note="Description of Artificial Sequence: Synthetic polynucleotide"
cagtcagtcctgactcagccccctagcgtcagcggcgctcccggtcagagagtgactattagctgcaccggctctagctctaatatcggcgctggctatagcgtgcactggtatcagcagctgcccggcaccgcccctaagctgctgatctacggtcagtcagagcggcctagcggcgtgcccgataggtttagcggctctaagtcaggcactagcgctagtctggctatcaccggcctgcaggctgaggacgaggccgactactactgtcagtcctgggactctagtcagaccctggtggtgttcggcggaggcactaagctgaccgtgctg

SEQ ID NO: 47 - protein, 217 aa, Artificial Sequence
  source: /note="Description of Artificial Sequence: Synthetic polypeptide"
QSVLTQPPSVSGAPGQRVTISCTGSSSNIGAGYSVHWYQQLPGTAPKLLIYGQSERPSGVPDRFSGSKSGTSASLAITGLQAEDEADYYCQSWDSSQTLVVFGGGTKLTVLGQPKAAPSVTLFPPSSEELQANKATLVCLISDFYPGAVTVAWKADSSPVKAGVETTTPSKQSNNKYAASSYLSLTPEQWKSHRSYSCQVTHEGSTVEKTVAPTECS

SEQ ID NO: 48 - DNA, 651 bp, Artificial Sequence
  source: /note="Description of Artificial Sequence: Synthetic polynucleotide"
cagtcagtcctgactcagccccctagcgtcagcggcgctcccggtcagagagtgactattagctgcaccggctctagctctaatatcggcgctggctatagcgtgcactggtatcagcagctgcccggcaccgcccctaagctgctgatctacggtcagtcagagcggcctagcggcgtgcccgataggtttagcggctctaagtcaggcactagcgctagtctggctatcaccggcctgcaggctgaggacgaggccgactactactgtcagtcctgggactctagtcagaccctggtggtgttcggcggaggcactaagctgaccgtgctgggtcagcctaaggctgcccccagcgtgaccctgttcccccccagcagcgaggagctgcaggccaacaaggccaccctggtgtgcctgatcagcgacttctacccaggcgccgtgaccgtggcctggaaggccgacagcagccccgtgaaggccggcgtggagaccaccacccccagcaagcagagcaacaacaagtacgccgccagcagctacctgagcctgacccccgagcagtggaagagccacaggtcctacagctgccaggtgacccacgagggcagcaccgtggaaaagaccgtggccccaaccgagtgcagc

SEQ ID NO: 49 - protein, 5 aa, Artificial Sequence
  source: /note="Description of Artificial Sequence: Synthetic peptide"
SYVVH

SEQ ID NO: 50 - protein, 19 aa, Artificial Sequence
  source: /note="Description of Artificial Sequence: Synthetic peptide"
RTRHSDMGYATSYAAPVKG

SEQ ID NO: 51 - protein, 10 aa, Artificial Sequence
  source: /note="Description of Artificial Sequence: Synthetic peptide"
VERSKSGFDN

SEQ ID NO: 52 - protein, 7 aa, Artificial Sequence
  source: /note="Description of Artificial Sequence: Synthetic peptide"
GFTFSSY

SEQ ID NO: 53 - protein, 8 aa, Artificial Sequence
  source: /note="Description of Artificial Sequence: Synthetic peptide"
RHSDMGYA

SEQ ID NO: 54 - protein, 10 aa, Artificial Sequence
  source: /note="Description of Artificial Sequence: Synthetic peptide"
VERSKSGFDN

SEQ ID NO: 55 - protein, 121 aa, Artificial Sequence
  source: /note="Description of Artificial Sequence: Synthetic polypeptide"
QVQLVESGGGLVKPGGSLRLSCAASGFTFSSYVVHWVRQAPGKGLEWVGRTRHSDMGYATSYAAPVKGRFTISRDDSKNTLYLQMNSLKTEDTAVYYCARVERSKSGFDNWGQGTLVTVSS

SEQ ID NO: 56 - DNA, 363 bp, Artificial Sequence
  source: /note="Description of Artificial Sequence: Synthetic polynucleotide"
caggtgcagctggtggaatcaggcggcggactggtcaagcctggcggtagcctgagactgagctgcgctgctagtggcttcaccttctctagctacgtggtgcactgggtcagacaggcccctggtaaaggcctggagtgggtcggacggactagacactcagatatgggctacgctactagctacgccgctcccgtgaagggccggttcactatctctagggacgactctaagaacaccctgtacctgcagatgaatagcctgaaaaccgaggacaccgccgtctactactgcgctagagtggaacggtctaagtcaggcttcgataactggggtcagggcaccctggtcaccgtgtctagc

SEQ ID NO: 57 - protein, 451 aa, Artificial Sequence
  source: /note="Description of Artificial Sequence: Synthetic polypeptide"
QVQLVESGGGLVKPGGSLRLSCAASGFTFSSYVVHWVRQAPGKGLEWVGRTRHSDMGYATSYAAPVKGRFTISRDDSKNTLYLQMNSLKTEDTAVYYCARVERSKSGFDNWGQGTLVTVSSASTKGPSVFPLAPSSKSTSGGTAALGCLVKDYFPEPVTVSWNSGALTSGVHTFPAVLQSSGLYSLSSVVTVPSSSLGTQTYICNVNHKPSNTKVDKRVEPKSCDKTHTCPPCPAPELLGGPSVFLFPPKPKDTLMISRTPEVTCVVVDVSHEDPEVKFNWYVDGVEVHNAKTKPREEQYNSTYRVVSVLTVLHQDWLNGKEYKCKVSNKALPAPIEKTISKAKGQPREPQVYTLPPSREEMTKNQVSLTCLVKGFYPSDIAVEWESNGQPENNYKTTPPVLDSDGSFFLYSKLTVDKSRWQQGNVFSCSVMHEALHNHYTQKSLSLSPGK

SEQ ID NO: 58 - DNA, 1353 bp, Artificial Sequence
  source: /note="Description of Artificial Sequence: Synthetic polynucleotide"
caggtgcagctggtggaatcaggcggcggactggtcaagcctggcggtagcctgagactgagctgcgctgctagtggcttcaccttctctagctacgtggtgcactgggtcagacaggcccctggtaaaggcctggagtgggtcggacggactagacactcagatatgggctacgctactagctacgccgctcccgtgaagggccggttcactatctctagggacgactctaagaacaccctgtacctgcagatgaatagcctgaaaaccgaggacaccgccgtctactactgcgctagagtggaacggtctaagtcaggcttcgataactggggtcagggcaccctggtcaccgtgtctagcgctagcactaagggcccaagtgtgtttcccctggcccccagcagcaagtctacttccggcggaactgctgccctgggttgcctggtgaaggactacttccccgagcccgtgacagtgtcctggaactctggggctctgacttccggcgtgcacaccttccccgccgtgctgcagagcagcggcctgtacagcctgagcagcgtggtgacagtgccctccagctctctgggaacccagacctatatctgcaacgtgaaccacaagcccagcaacaccaaggtggacaagagagtggagcccaagagctgcgacaagacccacacctgccccccctgcccagctccagaactgctgggagggccttccgtgttcctgttcccccccaagcccaaggacaccctgatgatcagcaggacccccgaggtgacctgcgtggtggtggacgtgtcccacgaggacccagaggtgaagttcaactggtacgtggacggcgtggaggtgcacaacgccaagaccaagcccagagaggagcagtacaacagcacctacagggtggtgtccgtgctgaccgtgctgcaccaggactggctgaacggcaaagaatacaagtgcaaagtctccaacaaggccctgccagccccaatcgaaaagacaatcagcaaggccaagggccagccacgggagccccaggtgtacaccctgccccccagccgggaggagatgaccaagaaccaggtgtccctgacctgtctggtgaagggcttctaccccagcgatatcgccgtggagtgggagagcaacggccagcccgagaacaactacaagaccacccccccagtgctggacagcgacggcagcttcttcctgtacagcaagctgaccgtggacaagtccaggtggcagcagggcaacgtgttcagctgcagcgtgatgcacgaggccctgcacaaccactacacccagaagtccctgagcctgagccccggcaag

SEQ ID NO: 59 - protein, 14 aa, Artificial Sequence
  source: /note="Description of Artificial Sequence: Synthetic peptide"
TGSSSNIGAGYSVH

SEQ ID NO: 60 - protein, 7 aa, Artificial Sequence
  source: /note="Description of Artificial Sequence: Synthetic peptide"
GQSERPS

SEQ ID NO: 61 - protein, 11 aa, Artificial Sequence
  source: /note="Description of Artificial Sequence: Synthetic peptide"
QSWDSSQTLVV

SEQ ID NO: 62 - protein, 10 aa, Artificial Sequence
  source: /note="Description of Artificial Sequence: Synthetic peptide"
SSSNIGAGYS

SEQ ID NO: 63 - protein, 3 aa, Artificial Sequence
  source: /note="Description of Artificial Sequence: Synthetic peptide"
GQS

SEQ ID NO: 64 - protein, 8 aa, Artificial Sequence
  source: /note="Description of Artificial Sequence: Synthetic peptide"
WDSSQTLV

SEQ ID NO: 65 - protein, 111 aa, Artificial Sequence; identical to SEQ ID NO: 45
  source: /note="Description of Artificial Sequence: Synthetic polypeptide"

SEQ ID NO: 66 - DNA, 333 bp, Artificial Sequence; identical to SEQ ID NO: 46
  source: /note="Description of Artificial Sequence: Synthetic polynucleotide"

SEQ ID NO: 67 - protein, 217 aa, Artificial Sequence; identical to SEQ ID NO: 47
  source: /note="Description of Artificial Sequence: Synthetic polypeptide"

SEQ ID NO: 68 - DNA, 651 bp, Artificial Sequence; identical to SEQ ID NO: 48
  source: /note="Description of Artificial Sequence: Synthetic polynucleotide"

SEQ ID NO: 69 - protein, 5 aa, Artificial Sequence
  source: /note="Description of Artificial Sequence: Synthetic peptide"
SYVVH

SEQ ID NO: 70 - protein, 19 aa, Artificial Sequence
  source: /note="Description of Artificial Sequence: Synthetic peptide"
RIRLETHGYAAEYAASVKG

SEQ ID NO: 71 - protein, 10 aa, Artificial Sequence
  source: /note="Description of Artificial Sequence: Synthetic peptide"
VERSKSGFDN

SEQ ID NO: 72 - protein, 7 aa, Artificial Sequence
  source: /note="Description of Artificial Sequence: Synthetic peptide"
GFTFSSY

SEQ ID NO: 73 - protein, 8 aa, Artificial Sequence
  source: /note="Description of Artificial Sequence: Synthetic peptide"
RLETHGYA

SEQ ID NO: 74 - protein, 10 aa, Artificial Sequence
  source: /note="Description of Artificial Sequence: Synthetic peptide"
VERSKSGFDN

SEQ ID NO: 75 - protein, 121 aa, Artificial Sequence
  source: /note="Description of Artificial Sequence: Synthetic polypeptide"
QVQLVESGGGLVKPGGSLRLSCAASGFTFSSYVVHWVRQAPGKGLEWVGRIRLETHGYAAEYAASVKGRFTISRDDSKNTLYLQMNSLKTEDTAVYYCARVERSKSGFDNWGQGTLVTVSS

SEQ ID NO: 76 - DNA, 363 bp, Artificial Sequence
  source: /note="Description of Artificial Sequence: Synthetic polynucleotide"
caggtgcagctggtggaatcaggcggcggactggtcaagcctggcggtagcctgagactgagctgcgctgctagtggcttcaccttctctagctacgtggtgcactgggtcagacaggcccctggtaaaggcctggagtgggtcggacggattagactggaaactcacggctacgccgccgagtacgccgctagtgtgaagggccggttcactatctctagggacgactctaagaacaccctgtacctgcagatgaatagcctgaaaaccgaggacaccgccgtctactactgcgctagagtggaacggtctaagtcaggcttcgataactggggtcagggcaccctggtcaccgtgtctagc

SEQ ID NO: 77 - protein, 451 aa, Artificial Sequence
  source: /note="Description of Artificial Sequence: Synthetic polypeptide"
QVQLVESGGGLVKPGGSLRLSCAASGFTFSSYVVHWVRQAPGKGLEWVGRIRLETHGYAAEYAASVKGRFTISRDDSKNTLYLQMNSLKTEDTAVYYCARVERSKSGFDNWGQGTLVTVSSASTKGPSVFPLAPSSKSTSGGTAALGCLVKDYFPEPVTVSWNSGALTSGVHTFPAVLQSSGLYSLSSVVTVPSSSLGTQTYICNVNHKPSNTKVDKRVEPKSCDKTHTCPPCPAPELLGGPSVFLFPPKPKDTLMISRTPEVTCVVVDVSHEDPEVKFNWYVDGVEVHNAKTKPREEQYNSTYRVVSVLTVLHQDWLNGKEYKCKVSNKALPAPIEKTISKAKGQPREPQVYTLPPSREEMTKNQVSLTCLVKGFYPSDIAVEWESNGQPENNYKTTPPVLDSDGSFFLYSKLTVDKSRWQQGNVFSCSVMHEALHNHYTQKSLSLSPGK

SEQ ID NO: 78 - DNA, 1353 bp, Artificial Sequence
  source: /note="Description of Artificial Sequence: Synthetic polynucleotide"
caggtgcagctggtggaatcaggcggcggactggtcaagcctggcggtagcctgagactgagctgcgctgctagtggcttcaccttctctagctacgtggtgcactgggtcagacaggcccctggtaaaggcctggagtgggtcggacggattagactggaaactcacggctacgccgccgagtacgccgctagtgtgaagggccggttcactatctctagggacgactctaagaacaccctgtacctgcagatgaatagcctgaaaaccgaggacaccgccgtctactactgcgctagagtggaacggtctaagtcaggcttcgataactggggtcagggcaccctggtcaccgtgtctagcgctagcactaagggcccaagtgtgtttcccctggcccccagcagcaagtctacttccggcggaactgctgccctgggttgcctggtgaaggactacttccccgagcccgtgacagtgtcctggaactctggggctctgacttccggcgtgcacaccttccccgccgtgctgcagagcagcggcctgtacagcctgagcagcgtggtgacagtgccctccagctctctgggaacccagacctatatctgcaacgtgaaccacaagcccagcaacaccaaggtggacaagagagtggagcccaagagctgcgacaagacccacacctgccccccctgcccagctccagaactgctgggagggccttccgtgttcctgttcccccccaagcccaaggacaccctgatgatcagcaggacccccgaggtgacctgcgtggtggtggacgtgtcccacgaggacccagaggtgaagttcaactggtacgtggacggcgtggaggtgcacaacgccaagaccaagcccagagaggagcagtacaacagcacctacagggtggtgtccgtgctgaccgtgctgcaccaggactggctgaacggcaaagaatacaagtgcaaagtctccaacaaggccctgccagccccaatcgaaaagacaatcagcaaggccaagggccagccacgggagccccaggtgtacaccctgccccccagccgggaggagatgaccaagaaccaggtgtccctgacctgtctggtgaagggcttctaccccagcgatatcgccgtggagtgggagagcaacggccagcccgagaacaactacaagaccacccccccagtgctggacagcgacggcagcttcttcctgtacagcaagctgaccgtggacaagtccaggtggcagcagggcaacgtgttcagctgcagcgtgatgcacgaggccctgcacaaccactacacccagaagtccctgagcctgagccccggcaag

SEQ ID NO: 79 - protein, 14 aa, Artificial Sequence
  source: /note="Description of Artificial Sequence: Synthetic peptide"
TGSSSNIGAGYSVH

SEQ ID NO: 80 - protein, 7 aa, Artificial Sequence
  source: /note="Description of Artificial Sequence: Synthetic peptide"
GQSERPS

SEQ ID NO: 81 - protein, 11 aa, Artificial Sequence
  source: /note="Description of Artificial Sequence: Synthetic peptide"
QSWDSSQTLVV

SEQ ID NO: 82 - protein, 10 aa, Artificial Sequence
  source: /note="Description of Artificial Sequence: Synthetic peptide"
SSSNIGAGYS

SEQ ID NO: 83 - protein, 3 aa, Artificial Sequence
  source: /note="Description of Artificial Sequence: Synthetic peptide"
GQS

SEQ ID NO: 84 - protein, 8 aa, Artificial Sequence
  source: /note="Description of Artificial Sequence: Synthetic peptide"
WDSSQTLV

SEQ ID NO: 85 - protein, 111 aa, Artificial Sequence; identical to SEQ ID NO: 45
  source: /note="Description of Artificial Sequence: Synthetic polypeptide"

SEQ ID NO: 86 - DNA, 333 bp, Artificial Sequence; identical to SEQ ID NO: 46
  source: /note="Description of Artificial Sequence: Synthetic polynucleotide"

SEQ ID NO: 87 - protein, 217 aa, Artificial Sequence; identical to SEQ ID NO: 47
  source: /note="Description of Artificial Sequence: Synthetic polypeptide"

SEQ ID NO: 88 - DNA, 651 bp, Artificial Sequence; identical to SEQ ID NO: 48
  source: /note="Description of Artificial Sequence: Synthetic polynucleotide"

SEQ ID NO: 89 - protein, 139 aa, Homo sapiens
SASSRRRQQSRNRSTQSQDVARVSSASDYNSSELKTACRKHELYVSFQDLGWQDWIIAPKGYAANYCDGECSFPLNAHMNATNHAIVQTLVHLMNPEYVPKPCCAPTKLNAISVLYFDDNSNVILKKYRNMVVRACGCH

SEQ ID NO: 90 - protein, 139 aa, Homo sapiens
STGSKQRSQNRSKTPKNQEALRMANVAENSSSDQRQACKKHELYVSFRDLGWQDWIIAPEGYAAYYCEGECAFPLNSYMNATNHAIVQTLVHFINPETVPKPCCAPTQLNAISVLYFDDSSNVILKKYRNMVVRACGCH

SEQ ID NO: 91 - protein, 138 aa, Homo sapiens
AANKRKNQNRNKSSSHQDSSRMSSVGDYNTSEQKQACKKHELYVSFRDLGWQDWIIAPEGYAAFYCDGECSFPLNAHMNATNHAIVQTLVHLMFPDHVPKPCCAPTKLNAISVLYFDDSSNVILKKYRNMVVRSCGCH

SEQ ID NO: 92 - protein, 15 aa, Homo sapiens
QTLVHLMNPEYVPKP

SEQ ID NO: 93 - protein, 15 aa, Homo sapiens
QTLVHFINPETVPKP

SEQ ID NO: 94 - protein, 15 aa, Homo sapiens
QTLVHLMFPDHVPKP

SEQ ID NO: 95 - protein, 13 aa, Homo sapiens
VSSASDYNSSELK

SEQ ID NO: 96 - protein, 6 aa, Artificial Sequence
  source: /note="Description of Artificial Sequence: Synthetic 6xHis tag"
HHHHHH